European Patent Specification EP 3 500 678 B1, published January 21, 2026. Title: VECTOR. Applicant: Autolus Ltd. The sequence listing filed with the application follows.

SEQUENCE LISTING (65 sequences)

SEQ ID NO: 1 - protein, 363 aa, Hepatitis C virus
ETHVTGGSAGRTTAGLVGLLTPGAKQNIQLINTNGSWHINSTALNCNESLNTGWLAGLFYQHKFNSSGCPERLASCRRLTDFAQGWGPISYANGSGLDERPYCWHYPPRPCGIVPAKSVCGPVYCFTPSPVVVGTTDRSGAPTYSWGANDTDVFVLNNTRPPLGNWFGCTWMNSTGFTKVCGAPPCVIGGVGNNTLLCPTDCFRKHPEATYSRCGSGPWITPRCMVDYPYRLWHYPCTINYTIFKVRMYVGGVEHRLEAACNWTRGERCDLEDRDRSELSPLLLSTTQWQVLPCSFTTLPALSTGLIHLHQNIVDVQYLYGVGSSIASWAIKWEYVVLLFLLLADARVCSCLWMMLLISQAEA

SEQ ID NO: 2 - protein, 476 aa, Artificial Sequence
  pregnancy specific glycoprotein (PSG) sequence, PSG17
MEVSSELLSNGCTPWQRVLLTASLLSCCLLPTTARVTVEFLPPQVVEGENVLLRVDNLPENLLGFVWYKGVASMKLGIALYSLQYNVSVTGLKHSGRETLHRNGSLWIQNVTSEDTGYYTLRTVSQRGELVSDTSIFLQVYSSLFICERPTTLVPPTIELVPASVAEGGSVLFLVHNLPEYLISLTWYKGAVVFNKLEIARYRTAKNSSVLGPAHSGRETVFSNGSLLLQNVTWKDTGFYTLRTLNRYPRIELAHIYLQVDTSLSSCCHPLDSPQLSIDPLPPHAAEGGRVLLQVHNLPEDVQTFSWYKGVYSTILFQIAKYSIATKSIIMGYARSRRETVYTNGSLLLQDVTEKDSGVYTLITTDSNMGVETAHVQVNVHKLATQPVIKATDSTVRVQGSVIFTCFSDNTGVSIRWLFNNQRLQLTERMTLSPSKCQLWIRTVRKEDAGEYQCEAFNPVSSKTSLPVILAVMIEI

SEQ ID NO: 3 - protein, 515 aa, Artificial Sequence
  PSG17 sequence with added transmembrane region
MEVSSELLSNGCTPWQRVLLTASLLSCCLLPTTARVTVEFLPPQVVEGENVLLRVDNLPENLLGFVWYKGVASMKLGIALYSLQYNVSVTGLKHSGRETLHRNGSLWIQNVTSEDTGYYTLRTVSQRGELVSDTSIFLQVYSSLFICERPTTLVPPTIELVPASVAEGGSVLFLVHNLPEYLISLTWYKGAVVFNKLEIARYRTAKNSSVLGPAHSGRETVFSNGSLLLQNVTWKDTGFYTLRTLNRYPRIELAHIYLQVDTSLSSCCHPLDSPQLSIDPLPPHAAEGGRVLLQVHNLPEDVQTFSWYKGVYSTILFQIAKYSIATKSIIMGYARSRRETVYTNGSLLLQDVTEKDSGVYTLITTDSNMGVETAHVQVNVHKLATQPVIKATDSTVRVQGSVIFTCFSDNTGVSIRWLFNNQRLQLTERMTLSPSKCQLWIRTVRKEDAGEYQCEAFNPVSSKTSLPVILAVMIEIYIWAPLAGTCGVLLLSLVITLYCNHRNRRRVCKCPRPVV

SEQ ID NO: 4 - protein, 183 aa, Artificial Sequence
  OX40L sequence
MERVQPLEENVGNAARPRFERNKLLLVASVIQGLGLLLCFTYICLHFSALQVSHRYPRIQSIKVQFTEYKKEKGFILTSQKEDEIMKVQNNSVIINCDGFYLISLKGYFSQEVNISLHYQKDEEPLFQLKKVRSVNSLMVASLTYKDKVYLNVTTDNTSLDDFHVNGGELILIHQNPGEFCVL

SEQ ID NO: 5 - protein, 302 aa, Artificial Sequence
  inducible costimulatory ligand (ICOS-L) sequence
MRLGSPGLLFLLFSSLRADTQEKEVRAMVGSDVELSCACPEGSRFDLNDVYVYWQTSESKTVVTYHIPQNSSLENVDSRYRNRALMSPAGMLRGDFSLRLFNVTPQDEQKFHCLVLSQSLGFQEVLSVEVTLHVAANFSVPVVSAPHSPSQDELTFTCTSINGYPRPNVYWINKTDNSLLDQALQNDTVFLNMRGLYDVVSVLRIARTPSVNIGCCIENVLLQQNLTVGSQTGNDIGERDKITENPVSTGEKNAATWSILAVLCLLVVVAVAIGWVCRDRCLQHSYAGAWAVSPETELTGHV

SEQ ID NO: 6 - protein, 254 aa, Artificial Sequence
  41BBL sequence
MEYASDASLDPEAPWPPAPRARACRVLPWALVAGLLLLLLLAAACAVFLACPWAVSGARASPGSAASPRLREGPELSPDDPAGLLDLRQGMFAQLVAQNVLLIDGPLSWYSDPGLAGVSLTGGLSYKEDTKELVVAKAGVYYVFFQLELRRVVAGEGSGSVSLALHLQPLRSAAGAAALALTVDLPPASSEARNSAFGFQGRLLHLSAGQRLGVHLHTEARARHAWQLTQGATVLGLFRVTPEIPAGLPSPRSE

SEQ ID NO: 7 - protein, 193 aa, Artificial Sequence
  CD70 sequence
MPEEGSGCSVRRRPYGCVLRAALVPLVAGLVICLVVCIQRFAQAQQQLPLESLGWDVAELQLNHTGPQQDPRLYWQGGPALGRSFLHGPELDKGQLRIHRDGIYMVHIQVTLAICSSTTASRHHPTTLAVGICSPASRSISLLRLSFHQGCTIASQRLTPLARGDTLCTNLTGTLLPSRNTDETFFGVQWVRP

SEQ ID NO: 8 - protein, 7 aa, Artificial Sequence
  complementarity-determining region (CDR) CDRH1 of OKT3
GYTFTRY

SEQ ID NO: 9 - protein, 6 aa, Artificial Sequence
  CDRH2 of OKT3
NPSRGY

SEQ ID NO: 10 - protein, 10 aa, Artificial Sequence
  CDRH3 of OKT3
YYDDHYCLDY

SEQ ID NO: 11 - protein, 10 aa, Artificial Sequence
  CDRL1 of OKT3
SASSSVSYMN

SEQ ID NO: 12 - protein, 7 aa, Artificial Sequence
  CDRL2 of OKT3
DTSKLAS

SEQ ID NO: 13 - protein, 9 aa, Artificial Sequence
  CDRL3 of OKT3
QQWSSNPFT

SEQ ID NO: 14 - protein, 350 aa, Artificial Sequence
  OKT3-CD8STK-TM-A construct
METDTLLLWVLLLWVPGSTGQVQLQQSGAELARPGASVKMSCKASGYTFTRYTMHWVKQRPGQGLEWIGYINPSRGYTNYNQKFKDKATLTTDKSSSTAYMQLSSLTSEDSAVYYCARYYDDHYCLDYWGQGTTLTVSSSGGGGSGGGGSGGGGSQIVLTQSPAIMSASPGEKVTMTCSASSSVSYMNWYQQKSGTSPKRWIYDTSKLASGVPAHFRGSGSGTSYSLTISGMEAEDAATYYCQQWSSNPFTFGSGTKLEINRSDPTTTPAPRPPTPAPTIASQPLSLRPEACRPAAGGAVHTRGLDFACDIYIWAPLAGTCGVLLLSLVITLYCNHRNRRRVCKCPRPVV

SEQ ID NO: 15 - protein, 7 aa, Artificial Sequence
  CDRH1 of 15E8
GFSLTSY

SEQ ID NO: 16 - protein, 5 aa, Artificial Sequence
  CDRH2 of 15E8
WAGGS

SEQ ID NO: 17 - protein, 15 aa, Artificial Sequence
  CDRH3 of 15E8
DKRAPGKLYYGYPDY

SEQ ID NO: 18 - protein, 15 aa, Artificial Sequence
  CDRL1 of 15E8
RASESVEYYVTSLMQ

SEQ ID NO: 19 - protein, 7 aa, Artificial Sequence
  CDRL2 of 15E8
AASNVES

SEQ ID NO: 20 - protein, 9 aa, Artificial Sequence
  CDRL3 of 15E8
QQTRKVPST

SEQ ID NO: 21 - protein, 358 aa, Artificial Sequence
  15E8-CD8STK-TM-A construct
METDTLILWVLLLLVPGSTGQVQLKESGPGLVAPSQSLSITCTVSGFSLTSYGVHWVRQPPGKGLEWLGVIWAGGSTNYNSALMSRLSISKDNSKSQVFLKMNSLQTDDTAMYYCARDKRAPGKLYYGYPDYWGQGTTLTVSSGGGGSGGGGSGGGGSDIVLTQSPASLAVSLGQRATISCRASESVEYYVTSLMQWYQQKPGQPPKLLIYAASNVESGVPARFSGSGSGTDFSLNIHPVEEDDIAMYFCQQTRKVPSTFGGGTKLEIKRSDPTTTPAPRPPTPAPTIASQPLSLRPEACRPAAGGAVHTRGLDFACDIYIWAPLAGTCGVLLLSLVITLYCNHRNRRRVCKCPRPVV

SEQ ID NO: 22 - protein, 6 aa, Artificial Sequence
  CDRH1 of TGN1412
GYTFSY

SEQ ID NO: 23 - protein, 6 aa, Artificial Sequence
  CDRH2 of TGN1412
YPGNVN

SEQ ID NO: 24 - protein, 11 aa, Artificial Sequence
  CDRH3 of TGN1412
SHYGLDWNFDV

SEQ ID NO: 25 - protein, 10 aa, Artificial Sequence
  CDRL1 of TGN1412
HASQNIYVLN

SEQ ID NO: 26 - protein, 7 aa, Artificial Sequence
  CDRL2 of TGN1412
KASNLHT

SEQ ID NO: 27 - protein, 9 aa, Artificial Sequence
  CDRL3 of TGN1412
QQGQTYPYT

SEQ ID NO: 28 - protein, 351 aa, Artificial Sequence
  TGN1412-CD8STK-TM-A construct
METDTLILWVLLLLVPGSTGQVQLVQSGAEVKKPGASVKVSCKASGYTFTSYYIHWVRQAPGQGLEWIGCIYPGNVNTNYNEKFKDRATLTVDTSISTAYMELSRLRSDDTAVYFCTRSHYGLDWNFDVWGQGTTVTVSSGGGGSGGGGSGGGGSDIQMTQSPSSLSASVGDRVTITCHASQNIYVWLNWYQQKPGKAPKLLIYKASNLHTGVPSRFSGSGSGTDFTLTISSLQPEDFATYYCQQGQTYPYTFGGGTKVEIKRSDPTTTPAPRPPTPAPTIASQPLSLRPEACRPAAGGAVHTRGLDFACDIYIWAPLAGTCGVLLLSLVITLYCNHRNRRRVCKCPRPVV

SEQ ID NO: 29 - protein, 234 aa, Artificial Sequence
  spacer sequence, hinge-CH2CH3 of human IgG1
AEPKSPDKTHTCPPCPAPPVAGPSVFLFPPKPKDTLMIARTPEVTCVVVDVSHEDPEVKFNWYVDGVEVHNAKTKPREEQYNSTYRVVSVLTVLHQDWLNGKEYKCKVSNKALPAPIEKTISKAKGQPREPQVYTLPPSRDELTKNQVSLTCLVKGFYPSDIAVEWESNGQPENNYKTTPPVLDSDGSFFLYSKLTVDKSRWQQGNVFSCSVMHEALHNHYTQKSLSLSPGKKD

SEQ ID NO: 30 - protein, 46 aa, Artificial Sequence
  spacer sequence, human CD8 stalk
TTTPAPRPPTPAPTIASQPLSLRPEACRPAAGGAVHTRGLDFACDI

SEQ ID NO: 31 - protein, 20 aa, Artificial Sequence
  spacer sequence, human IgG1 hinge
AEPKSPDKTHTCPPCPKDPK

SEQ ID NO: 32 - protein, 185 aa, Artificial Sequence
  spacer sequence, CD2 ectodomain
KEITNALETWGALGQDINLDIPSFQMSDDIDDIKWEKTSDKKKIAQFRKEKETFKEKDTYKLFKNGTLKIKHLKTDDQDIYKVSIYDTKGKNVLEKIFDLKIQERVSKPKISWTCINTTLTCEVMNGTDPELNLYQDGKHLKLSQRVITHKWTTSLSAKFKCTAGNKVSKESSVEPVSCPEKGLD

SEQ ID NO: 33 - protein, 259 aa, Artificial Sequence
  spacer sequence, CD34 ectodomain
SLDNNGTATPELPTQGTFSNVSTNVSYQETTTPSTLGSTSLHPVSQHGNEATTNITETTVKFTSTSVITSVYGNTNSSVQSQTSVISTVFTTPANVSTPETTLKPSLSPGNVSDLSTTSTSLATSPTKPYTSSSPILSDIKAEIKCSGIREVKLTQGICLEQNKTSSCAEFKKDRGEGLARVLCGEEQADADAGAQVCSLLLAQSEVRPQCLLLVLANRTEISSKLQLMKKHQSDLKKLGILDFTEQDVASHQSYSQKT

SEQ ID NO: 34 - protein, 153 aa, Artificial Sequence
  IL2 sequence
MYRMQLLSCIALSLALVTNSAPTSSSTKKTQLQLEHLLLDLQMILNGINNYKNPKLTRMLTFKFYMPKKATELKHLQCLEEELKPLEEVLNLAQSKNFHLRPRDLISNINVIVLELKGSETTFMCEYADETATIVEFLNRWITFCQSIISTLT

SEQ ID NO: 35 - protein, 177 aa, Artificial Sequence
  IL7 sequence
MFHVSFRYIFGLPPLILVLLPVASSDCDIEGKDGKQYESVLMVSIDQLLDSMKEIGSNCLNNEFNFFKRHICDANKEGMFLFRAARKLRQFLKMNSTGDFDLHLLKVSEGTTILLNCTGQVKGRKPAALGEAQPTKSLEENKSLKEQKKLNDLCFLKRLLQEIKTCWNKILMGTKEH

SEQ ID NO: 36 - protein, 162 aa, Artificial Sequence
  IL15 sequence
MRISKPHLRSISIQCYLCLLLNSHFLTEAGIHVFILGCFSAGLPKTEANWVNVISDLKKIEDLIQSMHIDATLYTESDVHPSCKVTAMKCFLLELQVISLESGDASIHDTVENLIILANNSLSSNGNVTESGCKECEELEEKNIKEFLQSFVHIVQMFINTS

SEQ ID NO: 37 - protein, 271 aa, Artificial Sequence
  membrane-IL7 sequence
MAHVSFRYIFGLPPLILVLLPVASSDCDIEGKDGKQYESVLMVSIDQLLDSMKEIGSNCLNNEFNFFKRHICDANKEGMFLFRAARKLRQFLKMNSTGDFDLHLLKVSEGTTILLNCTGQVKGRKPAALGEAQPTKSLEENKSLKEQKKLNDLCFLKRLLQEIKTCWNKILMGTKEHSGGGSPAKPTTTPAPRPPTPAPTIASQPLSLRPEACRPAAGGAVHTRGLDFACDIYIWAPLAGTCGVLLLSLVITLYCNHRNRRRVCKCPRPVV

SEQ ID NO: 38 - protein, 256 aa, Artificial Sequence
  membrane-IL15 sequence
MGLVRRGARAGPRMPRGWTALCLLSLLPSGFMAGIHVFILGCFSAGLPKTEANWVNVISDLKKIEDLIQSMHIDATLYTESDVHPSCKVTAMKCFLLELQVISLESGDASIHDTVENLIILANNSLSSNGNVTESGCKECEELEEKNIKEFLQSFVHIVQMFINTSSPAKPTTTPAPRPPTPAPTIASQPLSLRPEACRPAAGGAVHTRGLDFACDIYIWAPLAGTCGVLLLSLVITLYCNHRNRRRVCKCPRPVV

SEQ ID NO: 39 - protein, 20 aa, Artificial Sequence
  self-cleaving peptide
RAEGRGSLLTCGDVEENPGP

SEQ ID NO: 40 - protein, 20 aa, Artificial Sequence
  self-cleaving peptide
QCTNYALLKLAGDVESNPGP

SEQ ID NO: 41 - protein, 8 aa, Artificial Sequence
  Biotin mimicking peptide, streptagII
WSHPQFEK

SEQ ID NO: 42 - protein, 15 aa, Artificial Sequence
  Biotin mimicking peptide, flankedccstreptag
AECHPQGPPCIEGRK

SEQ ID NO: 43 - protein, 8 aa, Artificial Sequence
  Biotin mimicking peptide, ccstreptag
CHPQGPPC

SEQ ID NO: 44 - protein, 15 aa, Artificial Sequence
  Biotin mimicking peptide, long nanotag
DVEAWLDERVPLVET

SEQ ID NO: 45 - protein, 9 aa, Artificial Sequence
  Biotin mimicking peptide, short nanotag
DVEAWLGAR

SEQ ID NO: 46 - protein, 8 aa, Artificial Sequence
  Biotin mimicking peptide, streptag
WRHPQFGG

SEQ ID NO: 47 - protein, 38 aa, Artificial Sequence
  Biotin mimicking peptide, SBP-tag
MDEKTTGWRGGHVVEGLAGELEQLRARLEHHPQGQREP

SEQ ID NO: 48 - protein, 36 aa, Artificial Sequence
  two StreptagII biotin mimics separated by a linker, StreptagII-d8-x2
WSHPQFEKSGGGGSPAPRPPTPAPTIASWSHPQFEK

SEQ ID NO: 49 - protein, 50 aa, Artificial Sequence
  two Flankedccstreptag separated by a linker, Flankedccstreptag-d8-x2
ECHPQGPPCIEGRKSSGGGGSPAPRPPTPAPTIASECHPQGPPCIEGRKS

SEQ ID NO: 50 - protein, 251 aa, Artificial Sequence
  glutathione S-transferase (GST) sequence
MGTSLLCWMALCLLGADHADAMSPILGYWKIKGLVQPTRLLLEYLEEKYEEHLYERDEGDKWRNKKFELGLEFPNLPYYIDGDVKLTQSMAIIRYIADKHNMLGGCPKERAEISMLEGAVLDIRYGVSRIAYSKDFETLKVDFLSKLPEMLKMFEDRLCHKTYLNGDHVTHPDFMLYDALDVVLYMDPMCLDAFPKLVCFKKRIEAIPQIDKYLKSSKYIAWPLQGWQATFGGGDHPPKSDLEVLFQGPLG

SEQ ID NO: 51 - protein, 17 aa, Artificial Sequence
  Rituximab-binding epitope sequence from CD20
CEPANPSEKNSPSTQYC

SEQ ID NO: 52 - protein, 10 aa, Artificial Sequence
  7-mer cyclic peptide, R15-C
ACPYANPSLC

SEQ ID NO: 53 - protein, 10 aa, Artificial Sequence
  7-mer cyclic peptide, R3-C
ACPYSNPSLC

SEQ ID NO: 54 - protein, 10 aa, Artificial Sequence
  7-mer cyclic peptide, R7-C
ACPFANPSTC

SEQ ID NO: 55 - protein, 10 aa, Artificial Sequence
  7-mer cyclic peptide, R8-, R12-, R18-C
ACNFSNPSLC

SEQ ID NO: 56 - protein, 10 aa, Artificial Sequence
  7-mer cyclic peptide, R14-C
ACPFSNPSMC

SEQ ID NO: 57 - protein, 10 aa, Artificial Sequence
  7-mer cyclic peptide, R16-C
ACSWANPSQC

SEQ ID NO: 58 - protein, 10 aa, Artificial Sequence
  7-mer cyclic peptide, R17-C
ACMFSNPSLC

SEQ ID NO: 59 - protein, 10 aa, Artificial Sequence
  7-mer cyclic peptide, R19-C
ACPFANPSMC

SEQ ID NO: 60 - protein, 10 aa, Artificial Sequence
  7-mer cyclic peptide, R2-C
ACWASNPSLC

SEQ ID NO: 61 - protein, 10 aa, Artificial Sequence
  7-mer cyclic peptide, R10-C
ACEHSNPSLC

SEQ ID NO: 62 - protein, 10 aa, Artificial Sequence
  7-mer cyclic peptide, R13-C
ACWAANPSMC

SEQ ID NO: 63 - protein, 12 aa, Artificial Sequence
  Rituximab mimetope sequence
QDKLTQWPKWLE

SEQ ID NO: 64 - protein, 16 aa, Artificial Sequence
  QBEnd10-binding epitope sequence
ELPTQGTFSNVSTNVS

SEQ ID NO: 65 - protein, 136 aa, Artificial Sequence
  tagging protein binding domain
CPYSNPSLCSGGGGSELPTQGTFSNVSTNVSPAKPTTTACPYSNPSLCSGGGGSPAPRPPTPAPTIASQPLSLRPEACRPAAGGAVHTRGLDFACDIYIWAPLAGTCGVLLLSLVITLYCNHRNRRRVCKCPRPVV